European Patent Specification EP 3 788 065 B1, published August 27, 2025. Title: METHODS OF IMPROVING ANEMIAS BY COMBINING AGENTS. Applicant: The Childrens Hospital of Philadelphia. The sequence listing filed with the application follows.

SEQUENCE LISTING (5 sequences)

SEQ ID NO: 1 - DNA, 51000 bp, Homo sapiens
tccttttctctttcttttcaagacagggtcttgctctgtcacccaggctggagtgcagcagcacagttatggctcactacagcctccaactccagggctcaagtgatcctcccacctcagcctccctagtagtgggatctgcaggtgtgcaccactatgcccagctaattaaaaaaaatttttttttgtacaaacagggtctcactatgttgactaggctggtctcaaactcctgggctgaagggatcctccctccttggcgtcccaaagtgctgggattacaggtgtgggggtaagccactgcacccagccacgtctgtgctttcaaacacctctctcagcattttgctgctgcttgcttattgccagcccctccccccaggccatgtcggatcgatggccaggtggccgccaggtctagaggacgtcgattgtgcaagatcggcttttcagactgtcgggctagcagcctgggctgggggcctgggccttttgaccttccaaaggacaggatggggtacagaggctaggatcggggtgtcttcaccccctacacaaacacactatccctgctctgtctcaagcatctgtccctcaggaagtttgcaaggtggggcccagggcctgggaagaggggagtttatggggaggaggcagagttgttggggctgggacgagggacagtgggcagggctatggtgttcggtctcagggtcagggtcaggcccatgggcaggggccaggactctggggagggccacaggagaaggtgagggaaggtaccccctaacccagaatcctaaccagcctgacagtgcgccctcctgccctggcccagccctggctctgcctggagatggtgctgtactgagctcatgcccagcccccatgggcaggggccttcacaccttaggacacaggggtgccccccacgcacatgtcagggaggtacctgcctactgctacaggcccccttagggagcacacgccagagagcatggggcatctacgtgcttgagacatgcgtgaggggccacacaggtaggcaccacacacatgccacctgtcattgcctggacttcagtgcacaggcacacctggccccgacacaccagcgtgtcaccatgagaagaggagaaacccgctctcggcgccccccacagtgctgggccttcgcacacgttgtttcccgttcatcaagaaggggcgaatttttttcattcgacagatggaagaagcaccgctcagaagtcagggaatctgcccaggttcctacaactaaaagggagccaggtagggctgaaaaccggcggtcacggcaaagcccgggcgcggggccctgtcccatcccagccaatccataagcatctcacacttcacacccgctgcacactccactcacacgcctcacactccacacatgcctcacgctccacacacacctcacactccacacacgtctcacactacacacacgcttcacactccacacatgcttcacactacatacaccttacactacacacacacctcacactatgcacacacctcacactaaacacatgcctcatattccacacatactgtgagcatgcacacacacacacacacagctgcacacacctctcatgctccatacacacctcacaccatacgtacctcaaagacacacacaccttacactgcacattcccagcacccacactgcacacacatgcacagtccatatgcccacacaacacacttcacacaccccccaccccacaccatacaaacctcacagacacacctctcacacaaatcttataccccacacacaatccctacgctccacacacacacacacacacacacacgcacattctacacatacataatctacacacacaaattccagactgtctctcttacacacacactctgggacccatatgcccacagcacacagcatctcaggcgtgcaccccgcattctggcctcaggatgtagactcgctgaaagtcagccttgtctgagacagacgcccgctgccctgcacgcaccctagaaagccctggctcccatccggcacttcggcacgcatatggctcaaacccatctccacagcaacgctgttccatagaacaacaacgcaggtcacacttgtgacttaacctgtctaatatccacatgcaacaaggggtgtggtggcccgcgcctgtaatcccagctacttgggaggctgaagcaggaggatcatgtgggcccaggagctccagaccagcctggcaacctaatgagaccctgtctctgaaaaaaaaaaaaacaagagagccagaagaaaattgcttttaataatacattttatttatcccatgatcaccagtgttatttcaacataaaatcaatataaaaattgttatcgcgttggttgacatcctgtttgcacttggccttggaaacctggtgtgcgtctcccccgtgcagcttttctcagttcagactgactcaagagccacgggtgaccagcggctaccgtcatggacagcacagcgctacggaaccaggtaggaattcatgctgcgtgcggtcgctcatgcctgtaatcctagcgttttgggaggtcgaggtgggtggaatcacttgaggtcaggagttcgagaccagcctggctaacatggtgaaaccccatctcttctaaaattatgaaaattagccgggcatggtggtgggcgctgtaatcccagctacctgggaggctgaggcaggagaattgcttgaacccgggaggcggaggttgcagtgagccgaaatcacaccactgcactctagcctgggtgacggagtgagactccatcttaaaaaaaaaaaaaaaaaaaaaaaagaacgaggtaggaattcaaataattcccagctaaacagaaaatagcatcaaaccccacccctgcctcccctttctcctctccagtccccagagtatatgggcccagcctccttttctctctctcaggccagcagctcctttagtctcgcctgtccaggtaagcacctggactcacccttgtgagcccctgcactcacctgcaccggcctctgcacagtccccagtccttggctgtccctacctcatgctctcggggaccaggggctgtaaccaggcaggcatgtcaccaggcaacgggcctcgggggagagctcagatctcccgcacctgcctgccagcctctggggtgcccatgcgggggtgggggaagatggggcggggcaggcactgccttctcctacctcctgcctgtttacctgtacttagtcacagtgctgtccaggacccagcaggaggagttccatggagcctgaggccacaggccacaggggacaagggccagacaccctggtcatggctctaggccattgatccagcctgggctggctgggtgggggtggggaggccttggcctggacaaacagaggctcctgaggcctgtgtgcaggcccggcacctatctgccgctcccaaaggtaagcgggggcctccaggacaggggaccgggatctataaatgacctagtgacagtgtccaccctaagagctgggcctggctccctgcagcctgagccacctaccctgctccgaggccaggcctgcagggcctcatcggccagagggtgatcagtgagcagaaggtgaggggcccacagagctggggaggggagggaccacgcagggtgacaccaggtgtgtggacaggcacagcatcagtgctgggtggttggtggcctgggattcaggtggcagggacaggaggaagggagaggccaccctacccctgcctcgcaggactggacatgctgccccctccacacccggtaccccacctgggccttctggtgtaggagacaggcccggagccccacattgcacctatgtactgacttaagcccaggaccctgggctcacaggctcagagttggcatgtatgtgtatgtgtgttcgtgtgtgtgtctgtgtaggaagggcgtgcatctatgaatttttgtgtcatgaatagatgtgcgtatatccctccgcgtgtctccatctgtgtacatctgtgggtctgtgagtgtgtttatatgtgtggaagggacccccacccagtcccccacactctcaggactctagggcctaatggtttcactgaaagatgcccctatggccctagcccagagtccctgctctgctctgctctgccctggctgagggacctcgggtaagtcatgttacctctctctacctcagtttccccagccattaaatagagtcagcaaagtaggcaccccaggctgttggaggctgcagtggagtttgcagcactgcccagcacagggctggcacatggtaggagttcatacgcagtggttgaatccggatctgcattgctgggggagtcgcggccccgccccaaggagctcagcctccagcaggcagacccgagaccctccaatggccagaagggcaggagggagtgaggagcaggtgccagggtggggtccatggtgctcagagctgggggactgcttcaggcccctgtggcaattggagcacagtccccgcttccaggagttcaatgtgaggggcaaagagagagtgcccacaggtaagctgcacatcgcgaggggcagccgccccttctagggcactctgggagagctgcgaagaggtgaggtctgaactgaggtgacaggggctgcataagagctggccaggttgggaggtgggggcccaggcagaaggaagagtgtggggacgcctggccgtgaacaagcactgacagggctcaaggtccacgagggctcttggtgccggctggctgctcttaatccataaatgtttgctaccatcccattgttaaaatttctcaccaatggaagtccagtgtccttggggtgcgacggggaaaagagagggtgggaaaaaaggaggcaggagaagttggccaggccacatatgcacacagcaccttggacttctgtagggaggaaggagctgggaccttgtcattcattcatttaacaattactgagtgtccgctgagtaccagactctgctctcatgcagcttacagacagggaggaggcagataaatgacatatttgcatatcaggcaatttaggcctctgtaattgctataaagaaaaatgcaggagagacgggagtgcccagggaaggcctctctggagaggtgacatctgaccctttggaggaggtaaaggagggagccacgaggccagcagaaaggaaaacatcccaggcccagcaaggagcaaacctcccattcagcaaagaggacaggaaaactgagaccctgggtctttagggactgtgttctaggtggatggaagccgtgcgaggcttgtgggcagggcacatggtgacaacacgcagtggccattgtgtgagaactcactgggtaggggggtgggtgattggctattgcaggagtcgaggtgacagatgacggtggcctggatgatggtgggagtcatggggggccaagaaggggctggctttggggggcatttggaaggtagggccacaggcttttccaaaggtgctggaccctgggaatgggggagccgttgtattataagatagtaaagacaagagtggcaccgtcatcttcacaactgtccactgcccctcctcctgctgggcaggaaacccaagaggatgggaatgaggtctcttagagtcaccatgtgccaccctgtcgccaccacagagcctggcaccaagcaggtgctagacaaagatagggtgactgagcattgaacctgggaccccacaggcccacaccattgtccatgccccagtgccaggcctcacaagtcctccttcctggaggcagcaagatagaaagccctgtaccaggggcctagagacttggcagtttcattcactcattctttctgatccttcactcatgtgacgggctgtgcggcgttccatggggaaccccagaggtgagcaagatgctggccctgcctgttctgtaggggacagaggcaagacccaaagccaaggcatattcttgatctgatcaagggctgcccaggggagggggcagcttaactagccaggggcccagaacccagtgcctggcaggtcgcctggtaagagttccccacagtccaggcagggggactcagctgcacaaaggcagggtctcgtgggcctggggcaccatgtgcatgatggaagttatagccacgaggagggtggacagcagcctggccatggagggtcttggatgtcgcagcaaggggtttggatgataagtggctgggagctgtgaaaggatcctgagcaggtgagcgattgagctggggagggaggatgcgctggaagacgcaatggaggcaggggacctagtgaggaggccgccccaggggtttgggtgggaagttatgatgagcccgggggaattaatttcccactactgccatttggaccatggcttgggtttttacagagggtgtcctgaaaatgagcctctctgtgctgctcaaagtcctcccagatggatgcgaggggcatttagagggaggcaaaatctgcatagagaaggacgcctggcttggaggatgagaggggaggggaggcccaccaagcaccccaccatgagctgcccctcttcgggcttcctctaatggacccacgacctgctccgagcctcagtttccctctctttacactgattatctgagaggtagtagggctcagtgatcagggcgtcactctgaagtcaatctgcttgactttgcagcctggctgtgctgctgaccagctgtgtgaccttagccaagctgctcaacctctctgtgccttgactctcccatctgtaaagtaggagtgatcagagtacctgtccccacaggatctgtgtaaggcttacatgagaaagtgcacataaagcaacagagacaattgaaataaatgtcacctgttaccacctctatgcccccgagtccccatggctctatgactcatcccaaaatagctcctttgtgatccagactcaagagtaaaacagggccaggtatggtggctcacatctgtaatctcaacacttcaggaggccaaggtgaggggatcgcttgaggccaggtgtttgagacctggtctctacaaaaaataaaactataaaattagccaggtgtgctggtgcacctgtagtcccagctacttgggaggctgaggtgggaggatcactcgaacccaggagttggaggctggggtgagctatgatcgtgctaccatactccagcctgggtgacagagtgagatcctgtcccttaaacaaaaggggtgcgacgggaatatggtgtcctcctctggcagagggaggggacgagggactgaaagaagggcaaggagccaacccatcacctgggatcttcccaatccagcaaaccttctcagattttgaggacagccacctcagtcagaggtggccagcccaggacagacaggcagctctgcgctggggactcaaacctgccatgtggcctcatgcaagagtctcagcaccctgttactggtctgtttcttgcctgtttctcactagggatgctgtgaacatttgaggaagtgggcggggctgtcccacccgttgccggacgtttaccatttaccattccctggccttggccccataaaagccagtagggcccactccacatgcaggaatgtcctagcttagttgtggagggggatgtcatgcccagtgagggtcccctgcagtccctcccttccttgtatctgatgggggccgctcaacagagtcactgtggcttgacaccaaagacccttagctgggaacgatgccaaggggagctggagggagccaggaagctgggagaagggccagggcccttcacatccacctgggaggactttgagcattactaaagagccccgtttttggaaacccgctgtgtaaaatcccaagatacagcccaaaggaagccccgcctgcatctggggtgcattttatttatttttttatgtttttttttttctcaagcagagtcttgctctgtcacccaggctggagtacaatggcatgatctcagctcactgcaacctcccctgaccaggttcaagtgattctcctgcctcagcctcccgagtagctgggattacaggtgcccaccaccacagccggctaatttttgtatttttcatagtgacagggtttcaccatattggccaggctgatctcgaactcctgacctcaggtgatccactcacctcagcctcccaaagtgttgggattacaggcgtgagccacggcacccggccctggggtgcattttaaagctacacggtatttatggatatagtaagaggagatgaacttcgcagtagtctggagcctttgctctcccggtgggtgggtcaaaggctttctctgtactgtggggaaacctgcgtcaaaggccaaatacattgggatgtttgcttgaaagggtctcaaaatagagttggaaccctggagcgtggagaggggcgacattcagttgctatttaatcatgatttgttaattaacagctcatttatgggaggcatcttagattcgtggaaaaagcagggagtcagacatctagactcaacctccacttccctgctgtgtgatcttgggcaagcggcttagcctctctgggcttcagggtttttttaatctgtaaaatgcgtctgggagtgaatgtcaggtattcaaatcacactgggaaaatggggctaggaaaagccctagactgagttagtgctagaacactctgggtctcagtttccttatctgttcaatgggtgcagaactggaggtttaagtgagataaagcaggtgaagtacccacgtggtgtgggctggaggaagaaaacatgggacaatggttccacatccctgggtgacctgaaaattaagtgtgagatgtctcatgagggcacgaaatgaatattagtttttgttcccttcctctgccacaagactttgagagcagaaaggtgagagagacggtactctgtgaaggaaggcaggtccccggcccagcgcagtgccagctcaggggattctggggcgggggctaagtgcatggactgtgtgggcgtggtgggaagctccgtgaaccagaaccaggagcaagaaacagcattccttgcgtggacgggaaatgagggcaagaggtcagatgtctacagaagtctgcaccccatgtacttcagttctgtctgtgggtgcagcctctagggaggtgggtgtttaggtactgagacctccgtctgtcctctgaccatagggaagccagtgggaagcaaaggtggggttcttgagccagacccagtccagctctggtgcctgccctctggtgcgagctgacctgagatgcacttccctcctctgtgagctgtctcggcacccacttgcagtcactgccgcctgatgttgttactcttccactccaaaaggcagggaagtcctgcttccgtgccccaccggtgctcagcagaggctcccttgcaaatgcgaggctgtttccaactttggtctgtttccctggcaggatgcccgtggccgaggccccccaggtggctggcgggcagggggacggaggtgatggcgaggaagcggagccggaggggatgttcaaggcctgtgaggactccaagagaaaagcccggggctacctccgcctggtgcccctgtttgtgctgctggccctgctcgtgctggcttcggcgggggtgctactctggtatttcctaggtaacgttgtgggaccgcctgggagaggcacctggggaggacttggggtgactgtagcaggcacagcaggacaggactgggttccaggctcagccgtgcttagcatattgctgtgtgaccttgggcaagtcacttctgttctctgggtctccctccctgtccttccagctggagatgctgtcagaccctggctccaggtcctatggctcgggtctgcttcctgcttgggcaaagtgccccaaagctccccaccaggtggggaaagtgggccctcctagcacccagttcttgtgagccagccagcccacagagcataaacatcgccttcccttgcctgcagtcctcctgggttgcccctgaggcttggagccaacccagccctaaagaaggaggcccagaggcaccaatggtacctggtaccaattagtgcctctgctcacttgagcctagcctaggttctcctctaggctggggaccacagctctatcccctctgggtctccagggtccagcatgaatgggggacggagcaggcagctggagagcagccagccttggggccctctgccatgtccttaattatggctggcccctccctgatgtcacagccctcagtcagtcccctggtgcccggggagcaattggcctgtgctctgggcccattcatccaggcctccgttcattcattcatggaataaatgctcttgagcatctattatctttctctaagattgatggagtctctcctcttccttctgcctttgacagtgggaagtaatggagaaaccaaatcggactgtgcctctacactgtacactgtagaaggcccattcatttgttcatttactcagtgccaagcacctcctgtgtgccaggttctggggatagcccctgtccttgtgatttagccaaggcatcagacctgacatttacgctaaagcatagcatgtgatgggacagaggaagctgagggctgggaagccacaggagggacaacccagatgcctgcgtgatcagaagcatcccattaaacatcctgcaaaggatagctagtgctcttactggctgaatctcctggtggaattccaggcctgttgaaagcaacctggggaccaactttgtagcagtggagagaaatccatgtaggcctagatccaaggggtcagggttgggagtgtctggaaccagcatctgggagtgacactattgggaaccccaggtctgacacgggcctgcttgcaatgacttatagtgattctacccagagttgagcaacgcaggcagtagacgccatgtgcatttcaccaccagcaggaagccagtgccccagatagcacagggctgtgggggcctcctcaggtagcgggctaattagtctacagggtaaaccacggggcactgggctggagggccaggaactcacctgccaattatttctctttgcagaggagtttaattccccctgattatgctcctggggtaaatcaccccccaccccaggagaggtgctccatggggctgaggacccaaggggtgagtgctcccaagcctctgctgggggaagccaactcccccacagagggattaagggttgaaggaggcactttgggagctgtttgaaagactcctcccgccttgaccaggctgtgctcctgggactgggcgctgggcaaggaagtggatcagagacacgccctgccctgtctggaagaggaggtgcacaagtgaccagtgacactggagcaggacaggccccaagcgaggaggacagcctggcccgaggagagggtgtggctggcttcctaaggatggtagcaggacccttaataccaccaaccatatttcctgggtcctttccctttcctgctctcccaggcaagagttttatgtgttctcaagcccccagcacccgcctgcccctgtctcctgcttcagtgagaaaacaaaacagcttagaagagaagccccatatatgttggcccacctgccctcccagctgcatcacgtgcactcctcctgggaccccgatcccgccccctctgcccacacaatggcccagcaccagcaaggatgccctctctcccccagtgtcccttggggtgcctcccccatttctctgctccttgaaagagctgtcagtccacacacccagtctctctgtgccctttccaacctggctccctctgccccccaactccaatggccattgtcaagctcgccaacatcccaggttgctaaatccaatgtccacttctcagtcatcattgcacttgacccgggggctcacccccacctccagaagccctttcctccctagactttgggccgccaccgggtcctttccgctcagcaggttgctttttctgtgtccctgctgatgggtggggcctctcctttctctctccacccgcttctttcgtgatctcatctgctacccttagcttcaagtgccctttataccctgataacacccacatttgcatttctagcctgggcctctcccttgagcttgtctctagagctgcccctgctcttcctcttaatgtctaaggagcatctcggaccctatgctttcagaccatgaggtctctgcataatttcccccagacctgtacctccaacatcccagtccaagaccacttctttctggcaccttccccttactcctttctttcttttccacccagccccactttgccagcaaacctggtcatctctaactccaaaacacatcaaaagcagctgacgccaatcacttcccaccctctcctctgccacagctggggccaggctctgtccccctggacatctctcccctggagccctgcaggcgtgtcctcgatgctctccctgcctctgccctgcctccttagagcctttctcaacagcagagggaccatttgataaagcaaacgaaatcctctaacttcgctgcttaaaacctcgcttggggccaggcgcgtggctcacgcccgtaatcccagcactttgggaggccgaggcagatggatcacctgaggtcaggagttcgagaccagcctgaccaatatgcagaaaccctgtctctactaaaaatacaaaattaaccgggcgtggtggtgcatgcctgtaatcccagctacttgcgaggctgaggcaggagaatcgcttgaacccgggaggcagaggttgtggtgagcggagattgagccattgcactccaagctaggcaacaagagcgaaactctgtctcaaaaacaaaacaaaacaaaaacaaaaagaaaacaaaaaaaccacctcccattcctcccatcttacccagggtgaaagcccgagtcctcccaggcctggaaagccctacccagcctctccccttccccatctcataccctcctgctgtcctgttgctcactctttgctgctcctgaaacacaccaggcctttgcacttgcccctgcctgggacattctttccacagatgtacatcaccttcttccctgacctccatatcgcagcccgtcccatgccctgattcccaccgcactgaccacctctaacctgttatacacgatgtgtggtttaccgtctgattccttgctagtctacaagctattaagggcagttttttcttgatagttctgtccgttgttttgctcatatagtcccaagtactttggctcagttcctacacatagcaggctctcaagaggtatttactgagtaaatggataggggtgtaaaccagggctgtgagtctaccctcttcacttcagccaaaatagcctttgcaaaacagaagtctgatgacatcattcctgattttaaacttttcatggttacccttgttcatcgggtaaagacccaatgggccctgccctgcggaggccccagctccttgccgcccctccccatctctgactgctccagccaaacaggctttcagcccgggtcctcaccatggtccccgtgctaccggccccgtgccccatgctgctccctctgctggaaggtacttccctccctcttctcttaccaatttacagtttccccatccctacatctcagctggagggtcactccactctggcccaggctgagtgtcctcgtcacatcccctcaacagcaccatgtggcactgctccctgatggcactgcccacagacagatgccacatgctgtgtggttgccagagccacgcctttcttacccaccactgtcagcttcacaaggggaggcacatctgtcttggttaactggcgtaccccatgtagtaggtggttagcacacactgtgggatccctgggtgacctcacgagtggaaggatgcctagtggtgctgacccatgaccttggcctcctgggcctatgtggatttcctggccttcatgtcattggtgtcctggactggtcactgtgtcagcctctccctgggaacctgtaggacaccatccatctgggagcctttcacctccctggtaccttgcagccagtttgtcatccaataaactttagatgaccatgatgacaatgggagtgacaaagatgatgatgatgacattgatggtgccatggagacccaagacactgaggctgagctgagggtgtgggtggcaggagaaggcatggaagagacaggagactttcccacctgcttcctccactaaccctgctggttccttcctgggcagggtacaaggcggaggtgatggtcagccaggtgtactcaggcagtctgcgtgtactcaatcgccacttctcccaggatcttacccgccgggaatctagtgccttccgcagtgaaaccgccaaagcccagaagatggtaggaaaggatctgggggatgagagggagggaatatgggggtgaaaagagaggggtggggtctgatcacatggagccagttggtcaacccatctggagcattcacagggaccacagccctgctccaggcaccatggaagcagatgaggttgagggtcatgggaaagttagtggatgtttgggtcaatagcactcggattagatcctgatcatgcctcttaccaggggtggagcatgaccttgggaaaggtcccacagtgcagctgacactattgagggcccgctcctgcccctccgttacaggacggtggcccgctcctccccctccgttacaggacggtggcccgctcctccccctccgttacaggacggtggccgctcctgcccctccgttacaggacggtggccgctcctgcccctccgttacaggacggtggcccgctcctccccctccgttacaggacggtggccctctcctccccctccgttacaggacggtggccctctcctccccctccgtaacaggacggtggccctctcctccccctccgttacaggacggtggcccgctcttccccctccgttacaggacggtggccgctcctgcccctccgttacaggacggtggcccactcctgcccctccgttacaggacagtggccgctcctgcccctccgttacaggacggtggcccgctcctgcccctctgttacaagacggtggcccgctcctgcccctccgttacaggacggtggccactcctgcccctctgttacaggatggtggctcactgcacggaggctggtctactgcctgccactctcaggctgcaggaccactgcccagcaaggcaggccagaagtgccggggagttattcccaggagcaaccctgaaccatgagcgctggagtgggtggatcaataccgcagcttctttggccctggcagggggaatagttcacagaatgttccaggctgtctcccagagatgccctattcggctgagctcagatgctctcagctctacactgcgcattcatggccctgtgttggttgcccactttccagtctctccctcccaactactgtttcccagaatcacctccaaataaaccacttgccccaccttgtcaatggagggtctgcttctgagggacccagcctgaggctgcccgtttcctcctccatgaggtaggggtgataacaacaggacccggctgcagatttgttgtgggttgcagtgaagttgagataacacgaacactattcccacgctgcgcaaatgcttaagagcctgtaatcctgccagcagcgctgtagttggagatgcgcaaaaactacccatcagagctgctggcttgtcccaggccatgggaggaggtgcagaggggacccaggagccgagtggggtttctcagagttgaggagtgacttttggcaaggggcagaggggtcatcagcagtgcaggtggaggtgagagtcgggtgtagtggaaacagaaagaaggggatggggtgtgagattcatgcatgccccggcccggccactcagcactgtgtgaccgtgatcaagcctgtccaccttggagaatcatgcatggagcggggctgccagtaggagcaaagggcacctccaggtaggaagtgggcctgtctgccctgcagagggtcccaggggctgttgtcttcccttctcacagctcaaggagctcatcaccagcacccgcctgggaacttactacaactccagctccgtctattcctttgggtgagttgtccttgcccctgaccagctcctgcaagaagctgagattcaaagaatgggaggggcctctgtaggcttctgatgcaatgccttcatgtttcaaatggggaaactaaggcatagagagggaacttggcttcctgcatgtcaccctcccttcactgggctcatctgtagaatggaaacatgggtgtgataggtttgcaccagacaatgactgtgatggctgatcaagggcctgacaccatcaggcgaggcgatgttggaggggcatggggttaaaagcattggctccagggcccgactgccccgtccacatctggttctgctacttgcggcatagtttatgagacacaagttcacctctcatgcctcagttttctcattcgtaaaataaggattatgagagcgcctccttcagaggtcgctaggaggcttctgcgtgaagacggacagcaatggctgaggtgcggaaagtgctcgatgtgcatgagcaggggtggagctggggccagacctcagaatccttccctggcctctctcacttctgcctgccttagggagggacccctcacctgcttcttctggttcattctccaaatccccgagcaccgccggctgatgctgagccccgaggtggtgcaggcactgctggtggaggagctgctgtccacagtcaacagctcggctgccgtcccctacagggccgagtacgaagtggaccccgagggcctagtgatcctgggtcagtactgcgagtggaaacgtggggttggcctcatgaggttgggggaaacaagctgtggtgtggcccggggaggctgcctgccaggcctggggtgctgtcagggtgggccccccaggagagccccccaggtgaggtagcagtgccattgcattcaaggagccaggaaagaagggtgggatgggggcatttagggtaaatctcagacaaggctggctccaagggtctcctctaattttattttcattgtattttcttttctttttttttttttttgttcttgtttatttgtttgttcatttccttttatcagaagccagtgtgaaagacatagctgcattgaattccacgctgggtacgctatttttttttcccctccccattttccttttgagttggcatttgtcttgactttgttgtgtatcagggggacacatggcttctgttgtgtgtgcagggagccctggccaagagtcacccaggggatgccatggtggactcagcgatgtgtcccaagcaagtcttggagcctgtagggggagaggaggtggcgacgtgcatgcgtgtatttgtgtgtgtcttgtagacgggtgtgcatgcgttcctgtgtgggtgtgaggatgagtcaggtttagtggtccacgaacgtgactctcctctatcattcacttcaacctgcccacaagctagtttccactgatggtagaaaatcatcttgccaattcacggtttgtcagtcacgttggttttaaaacttggtcttttggaggtagcggtgccattgcattcaagaacgctccttccctcttttcctttccttcccagtcaggctcatcagccctccctccctacctggtgccgtattgctagagtcaccttgcatttctccaagcggacccacaatctttcagctgaccagcacagtcaccacgctgcacaaggcaggaggtgctgtccaagttgtagtttgtgtgagttgtgcagtgcaccaactggctgctggactctatggcccctaaattctcagattcctcccacactatctagtgttgtcacccagagccaaggtgggggtgagcgtctcaaccccttctcagggagggaggcagagtttaaatccttgttatacctttccttaccttcccgtcttcccatcctgctggtcaaatgcttgcttctttgttggatggaggtgatgaggtcaaagtacagttttcaaagaggtgaaatcatgattctcatacaaagatagagtgaccatgtgtcaaatatttatttggctgattaatgggggaacgagtagaatggtaaagaatgcaagaaactgatctatttgtctatctatctatctatctatctatcatctctgttgatatctgtctgcttgtctatctagttatctaactagctagctgtctattatctatctgtctgtctctctgtctctgtctgtctagctagctagctgtctgtttatatctatctatctatctatctatctatctatctatctatctatctatcatcaatcattaatggaaaaagagaattgctagaataagattaccaagttagatacaaacctggttaaggtcctaccaggcaagaaaactcaaacctttggagttgtcttttctagtgaattaaaatcattgacagcttattacagtcttctgaaagttaacatctacctctacagagtctgaggttgataatctacaaccaatagtaagtcagagatattactcctgagagcctcagggggacttaatcagatgatgcttggagacagagactggctcattgcagcctggacaccgaatctggtcaattgctgcctgattttgtatagcccatgagccaagaatgacatatatatatatataacagagtctcactctgtcatccaggctggagtgcagtgccgcgatcttggctcattgcaacctccacctcccaggttcaagcaattctcctgcttcagcctcctgagtagctgggactacaggtgcctgccaccatgcctggctaatttgtatatttttagaagagatgaggttttgccgtgttggccaggctggtctcgagctcctgacctcaggtgatccacctgcctccacctcccaaagtgctgggattacaggtgtgagccaccacgcctggctccataggccatttttcaattattaaaaaatataaaagtcagccaggcatggtggctcatgcctgtaacccagcactttgggaggcagaggcaggcagatcacctgaggtcaggagtttgagaccagcctggccaagaaggcgaaaccccgtctcttctaaaaatataaaaattagccgggcatggtggtgcgcacctgtagtcctaaccagtcaggaggctgaggcaggagaatcacttgaacccggaagatggagcttgcagtgagctgagattgtgaggttgtgccactgtactccagcctgggcgacagagtgagactccatctcaaaaaaaaaaaaaaaaaaaaaaaaaaaagaaagaaagaaaggaaaggaaaaggtcctatggaaagttattttttctcctgcaatagaagtgctatgtaatagcctcatgttgcctcgtgcctctgtgtccccatgttcctggcagttgttctgtaattatctgtgctcagtgggtgttcgtttcatgaatgaatgattgaacaaatgaatgaaagcatgaatgaggagactggttcagtgcatgtccagagcacagagtctcagggggcagagataacaactcaaatccttgaagtcgactttatgagcacttccttcatgccaggccccattcctgcgctgaggacaccaggatgaccgtgtcctcacccctgccctcggaggagctttaagccccatgagggagacagacacataaacagattctcataacaccaggtgccagtgtgagaatagaggccccagaggcagtggagagagggaattgttcgttccaaagcagaagagggggcaaatcaagagcctcacacagagtcccagatctacaggagggaggggttgctcctgactgggggatcctggaagacttcatggagggggcatcagatttgggcatgggccgggcgtggtggcacaagcctgtaatcccagcactttgggaggccaagttgagcggatcacctgaggtcaggagttcgaggccagcctggccaacatggcaaaaccccatctctactgaaaatacaaaattagctggtcatggtggcccatgcctgtaatcccagctacttgggaggctgaggcaggagaattgcttgaacccaggaggtggaggttgcagtgagccaagattgcaccattgcactccagcctgggcagcaagagcaaattccattaaaaaaaaaattagctggacatggtggtgtgcacctgtagtcctagctactcgggggtgggggtggggggctaaggtgggaggatcacccgagctcaggaggtcgaggctgcaatgagctgttgtgatcgcatcactgcgctccagcctgagtgacaggctgtctcaacaataaaataaaataattttcaaaagaaaaagaaattcaggcatgggggtaggcaggaatttgtcagggcgagaagaagaaagggttccctgagcagagggaatggcaggggcaaaggctgggggaggggaacacccaaggcgtgttcagttaattcctcccagccccgagaggtgccaggctccctgaaggtgtttctgattaacaagaggttagcacacacctctccacggaattcgtctcaaaaaaaaaaaaaagggtaattattaaagtggcaagagcaaagaatctgcttggagcaagatttaaagaacacaaaaccctaggaagagccagccatctttccccagctgctggtggaggccctgtcccttccctaggcagacattgttgttctctctctggggaggtcagctccccactgcagtcagcatggccaggggtcagggagaaggggctgagccacaggtggcagcatcagagcaaagtgtattcacctccattcccttcctggtcctcagcactgcccagaggaggtcataggacagggattattattacatccatttgacagaacttggaatggctaagccactggcccagactcagttaactacccagaggtagtgaacatctacctctacagagtctgaggttgataatctgcaaccaatagtaagtcagagttattactcctgagagcctcagggggacttaatcagacaatgattggggacagagactggctcactgcagcctggacaccgaatctggtccactgctgcctgattttgtatggcccatgagccaagaatgacatcatcacacagctgatgagtgttggtgctaggtggggagggtagtgcccctccctccttctctccagttccctccccatataccccctcccctgggggcccagcagatggcactagcctggggggcctgccctcaggctgaccaagctgacagggggacttttgcttgcctgtggccttccaaagaagacgatttaaagcagagaaaacagactgaaaactcaggttttataatttcatgtcaccaggctgcctcccacatcccaggttcattcctaaatccccactggctcctggaagaacaccaggcttctggcgaggtttaaatgagatactggatgctccacgggagagaacatgttcactggcagaccctggtgcctagatcgaacacacagtcggtgcacagtcactgttttgaatgaatgaatgaatgaatgaatgatgcaggtggtactgctttgtaagttctagcagtgcatcagagcttacggattagatggaagagcagagactcactggtgtgtggggtaggggggtggggtatgatggtgaaacagttgtgaagtgaggcagccgtgagatgggctaggtctgagcctcaggcggggccagctgcaggatgaaaagtcacaggcctttctccccagccctacctgctccgtctccctcacacccacctgaggaaccaggcactgcctttattgagcccctactgtgcaaggtgctgtgctgggcattcaaacgtgtatcatcctacagcctctgctggcggccctgcaagggtggtgttatcgtcccattctatagatgaggaaagcaaggcccaggaaagattaggtggtggctgggcaaacccagatgtgtctggcccaggtctgtgcaatggacacaatcattgaaagtatctcatacagctgttgtgggcattgagcgagacagtgagggaaggcattcagttcagtttctggcctgtagcaaatgcttgataagcacctgttttattctgatggcttcaccatcattagctcaaagctcatgtcctccccccagggcagcctcccagactcctccttagggcactcccttctctctaccggaagtgaagccctcatcccttcttctcctcattgcctgtggcctcgctggtctccacagcagccagaggagtgtgtggtccaagccagcccatgtccagccttgcccaaccttctgtggctccctatggctgcaggagaaagcagcgcccatcctcggaatggcctgggccaggcctccctgccttcagcttgtcctctagatacacgtgccctgtgtgtacttttctcaaagctgcccggctcgccccagcctctttgctcacgcagggacccccaggatgcccccagcccacaggccgggtttgaagccgtcacctcctgagctattcttgcctgttctgtgtctgtctgtccccgctgtcatccatgtccccaggcagcgactggatttttacctgggcactgagaaggcgtgaagctcagtgtgtgtccattccatgagtgaatgactgaaccaatgaacaaatgcatgaatgaggatactgacagggaaagagaaggatggggtagagcatgtctggctatccccacccggctcccctgcccagcccatcctgcctggtggaggaccttgagggacctggctccccagggtcccctccttctggctcacaggaatcaggggctgtgcccctctccccgctccaggttgttaccgctacagctacgtgggccagggccaggtcctccggctgaaggggcctgaccacctggcctccagctgcctgtggcacctgcagggccccaaggacctcatgctcaaactccggctggagtggacgctggcagagtgccgggaccgactggccatgtatgacgtggccgggcccctggagaagaggctcatcacctcgtgagtccctgggaaggagggcaggagggagggctggaaaagggagtggttgatgggggagttgaaagtcacacacagcattcttagacaagggagggtaggaccttgggcctgggtatctgggagacaggacggctagcttagaggggataggggagaggaggctggagatggttgtgtactgggggcgcttcccctccgcgagcctcagtttccccatctgtaacaaagccgttgttgtagatgactcctgaagtcagctctgggaggcaccgtggcttgttgggatgtttcagagtctggctgcagcctggactttcaacctctgggctcgttcctaaatcctgactgcttcctggtagaacacccaccctctctgcttcccaggcttctggtggggtttaaatgagatactagattccccatgggaggggatgtcttcactgccgggccctcgtgcctagaccaaacgcacagtaggtgtgcagtatctattttgagtgaacgaatgaatgatgtaggtggtactgctttgcaagttctagcaatgcatcagagctcacggattaaatgtaagagcagagaggcttactggtgtgtggggcgggggtgtggggatgtgacggggaaccccctgtctcctagctgcgtgccctaaggcaagttactttgcctcttagaacctgcttaccttgccggatcattggaggatttaaatcagactatctgtgccatgatccttacacatagtgagtgcctagcacttacacgctagccattattgttatcattatatatgctctaactgggactgggccgcaaaaggcattgagtgccaggagccatttggactttgatatttggtaagtggggagctattgaaagttcttgagcacagaagtagggctttagggcataagatatggagtggagtacagaagtgatcaggatcagagggcaggtggttgggggtggggaggagggactggaaatggccttgacctctgggagcctggtcctcccacaggatggggagatgggtgttagcctacaaagcactgcaggaggtggggaagatgctctgggctgggcagttctcagcgattgtttattgagcacttactttgtgctgggcgtcaggctgatgcctcttctgtctcacttgggctgtggccagcctccaggcagatggggatgggaccagtgtgttcagatcaagcgcagtctttgaatgtgagctggcagaggttcttgccacacccctcccccagggcctctccaagctgctctctccttgtcacccctcctgctgtcctgctgggtgtgacctcgatctgcggcatgtgcgtgggctgagtttctggagggctctgggaagtgcagagaagccagacaccatctgacttccaggtccaaaaagggtggggacacttaggggtttcccctggggcttctccaggtgcctctcagcctgggaggggacctgactgccaggcccagctctgttcctactcactgtggctcctggtggctctctcatcccagacccttggagaagctctaaaatgacaggtcagacaacatttggggttctcaagcttgtaccccagacacctgctagggaatgggggtgagggggactttggtggtgatgggaagacagagcaggtggccccttgctcagtttcaaccatgtgctttgattctgcgttccatatttcatttataagaagggctctgccgctaggtaaataaaataaaaccccccaacaatgaaagctaaagcccccattaaaggtgacctccaggtctcttccatcctaatatcgtatctcccacctcccagggaagatgagccggtaaggccaaaaaggacgtggctgtatgggagggtggggggcaccggtgtggttggggagacttgggtgctgcagcaggaagatcaagctggaatggtaggaagaagggacgagggcctggggggtgaggggggtggtgcctgctactggaggccacctccctcccctggcaagaggccaggggaaatgccccatccccggaccctgggcaccaagaccctcccagggagacccttggggttatgcccaccatgcctccagctggctgcaggctgcttgggtgccatgtgtagcgattttgaggctgtgcttggaggagctcaggtactcgcttgccaaggtgcctgaaatccctccagcagcaccccttcctcctgtcaaggcccaggtgcccacgcacagtctgcaggcagggaggctattgggttgcccattcagagggaggtggggccgttagtttcttataaattgacccatcagatgcgctggactccagagagtgttgccattgacactgggaagtttgggggaggttggtgagagggtgaaggggagctggggaacccctgtctgagacaggcagaccaggggcacctacatatgtgggagggtaccagccatcacagacagtgcctagcgcaggcctatctctgccatggactgccggtagggcctcagtttccctatctggaaatcaagcagctgaccccaacagtgtcaccagtcttttcagggctgacattccagatttctaaaagcccagaagtctaagatacggttatttgttccgagcctcccaggcgccaagctctgggcagatttctggggcaccctgggggtcacgagaccacacctgccttctccctgcctatccttgagcacagccaggagtcgcggtgccagaaacggtggtccctgcagatgccagtctagtcttcctgccagggacgctaggggtcacagatgattctgtagcagggtggaggggtctggggagggagcatgggactcgagccagccgtcatcatcaaactgtaagctccagaagtctggggaacctcctggcctctctcacccgaggagctagcctggtccttggagggccttcagtctgtcctctggggctggggagacacagaattctccccacagacacacagtggtctctggtaggagacccggacccagaacccagatgtccagactcccgtccaccctcccccagcagccgcctgccgccctccctgccactcccctcccagaccccagcccagccttgccacctttctgttctgccagggtgtacggctgcagccgccaggagcccgtggtggaggttctggcgtcgggggccatcatggcggtcgtctggaagaagggcctgcacagctactacgaccccttcgtgctctccgtgcagccggtggtcttccagggtgagaggtcaggggtccctggggcaggggaggggtggtggtagaatccaagggccctccactgggctcactgctcaccttttttgcccaaattgaggatgggatggggagagggaagattctggaagctcctgctgctctccactccccaccccggcccccctcttccttccgtcgtttgcacttccacccccctcttccccttgaccgtcctaccattcgcagtctctgtcttcctggcatcgctcccttgcttccctcctctttctctgtccttccttctctctccttttctcttttctgtgctgaccgcctctcctccctcctcactcgcctggacctgtgtcccctcccctctgcccctcaccccctccctgccctctccccttggcacccaccggtggctgggcctggaacacgggtctgtttgcagcaggactaagaactccttggattccgccctagacagtccgcttacagccaagagggcgcagggagcttggggaggtgtgatggcagcacagccaggccatggccactggtgtggcaggtctcccactgccttcccagcccccaccctcctcctgcttcgggacctccctccttgcccccttcccaggaagggcacgtcccaccccgcatgggacagctgtcctgggcctggaccagccatacttctgcgcaggaggcccaaactttgccatttctggagctcaggaggggaggatggcagagaggaggccatagagtgttggcagctgcttctgcctcacctctctccccactcttctccctcccactcagggtcccagccctcttctcggtttatccccaaactgtctggcatagacctgggtccccagctggccaaactggagcgctaaatgggtagcagagctgttcccttgggagtctgacacaggctcgaggcgggagggaacaaagggctttgggggccctggcccaatggagagatggccagggcaggtgagcatgctcctgtcctgacccctggacccctcagcctctcacggtgtagcctcaaccaagccactccttttctccgaacctcatcttggaaaaggggaacagctctctctcccccagccaccaccgtgaggcctgtgcaggtgtgaatgcattttgtaaactggcgagtgctgtcccgcaaatatcaataactaacacggatcgagcacttactacatgccaggctgtttgaatgtttatgtctttttaatccactctactaccctatgaggtgtgtgctattactgtcctcattttacagatgaggaaactgagacccagattcacacaatcacattcaaccacagcaatttgctggcagaggtggtaggggtggtggggttacaagctgcgccagcctgctgggaggtgcagccaggggacccctgtgtaacagctgctctcctggtccagcctgtgaagtgaacctgacgctggacaacaggctcgactcccagggcgtcctcagcaccccgtacttccccagctactactcgccccaaacccactgctcctggcacctcacggtgagaccccaccctgcctgcccacctgccctctgccgcaagcacactacaggtccctggtgacccgggatgagagggggcagtgtcccgcctctgctgaagcgcccacaggctgagccctgggtacacatcctgccagggtggagagggctgtgggcgaggtctccctctgtgggtcacagcaatgcctgtttgttgagtgactgacagactttagccccacctgggattctgtgtttccttctctttgttgttagggaggtgggttcaccaacctggccacaccccatgggccacctgatggcccgctcctccctcccaggtgccctctctggactacggcttggccctctggtttgatgcctatgcactgaggaggcagaagtatgatttgccgtgcacccagggccagtggacgatccagaacaggaggtaccacttcctctcctccctctggcttcctttcctccctccccctccctctcttccctcctcaatagtgaccccctcattggaagcccaagtccccaatctcagaggggcagcaaggggagcgagcagaggctggggctggtgtcaggcctgttgcccttgaccttgtcctcgtcccagcctccgccctggccccggcttcccctctggctaccccagaggtctcagacacgtttggtcatcagacaccttggatgtttattctaattacagcaaaattgtctcatcttcttgggtgctgtaaccccctctggcaccctcaatccttcaataaaatgtttccagagccaaaggactcatgggcactttggtgccttccctctaaacccaaggcgtaccatcagaggtgcctctcccttatcacgaacccctgctgcacagccaggcccaatcccattgcacagggtaacatggaaatcatgggtgccctggatcccccgaatccccaacggggcacttgccctcttccctgctcttgcccttgctccctctggtaactaagtttccgacaaagaagtgagtccttacagagatgtgagcaagagacagtggggttaggctaagcgactaccgttgccagggtcactatggcatgaggccagtaggtgcccactgggcctggccaccaggaagccatgggtggtgccgacagcttcagaggcctgggctgggcaaggaggcagggaaacagagacagggtgtatggacaggttttcatttgtctgggaagaaaagagaactaggaaattcaaggaaggggacatttaagacgggagaggttccatatctcaaatgtgtggatcatcccagcatccccagagggagagaaggaggctcaggtgcaggtaatattgtttagagtggggagggtgggcaaggggagagggaggccctcccatggctccattgttggggagcagaggtttggggagagagaagaggaatattgaagcagcgatggcagagccagggagaccctttccctgggaatccggggtgaaaacggtcatcgtgtcagcgtcaggaaagaggagactctatccttcatcgcaggttgggcctctgccctcccttccaacctcggaattctgggggcctaatgggttcagagtctagtatgaaagatttgtcatttcttgatttcacagagtttgaatatctaagatgccagtcttggaagatgccaaaattggaaggctctggggctctagaattcttggatttctggggtgtgtgttcccaatcaccaacacttgtaatttgcttgttggctgatcctattcaaaaggatcatccagacaaaaggtgacgaagaatgacaaggtttgcttgactcctttttgcaatttatctgggactaggattaaaagaaaggagaagaaatactcatggcatgatctagggctatgctgttgggggtaacatggggagtgactttgggcctgtgctgttgggggtgatatggcgaagcagtgccttcagggctttgcatttggtggtgatatgctgatggagtgtgacatcaggcctgtgctgctggggtgacatgctggttcagtgatgtcaggcctgtgctgtctggagagcagaaggcttctgtagcatgatgggggcacctctgggaacggctgccctgacccctcatggagctcacttgaagcctccttgctactcacctaggctggggatggctggcttcacccccgctcacaggaacccgcagggtgaccctgagatggatccatgattcacagttctgcgaatgatgagaacatgttttcctgcctccctccctaccgcagagctgaactttatgtctcagggaggcccacaaaggagaaggaacagtcttgggtctgacactccctgtctcatccctcacccccttggcgactccatttgccagaggcggggccccagcattcaggggttgtggggggttcggtggcctggagttaggtgctaagacaggcgttcagtgcattggcccaacaacttgtgtggtcattggcgccgttcctgtttcccagagaaggaaatcaaggctcagcaggattaggtggcacgcagatgggtccacagatggggtctctcccatacccccaacagccacaaacagcaggccaaaggatgctccaccccatgcttcctgtgggaaggccctcctccctccctgatgcagttgggcaagggtctgggtactggggagacagggacttcgtgagctacccttgggtaatgacagagagagtgtggaacacggatgggagagtcttttccctaatccaaaggaatgatgccttgatggtgaatttgaggcactaggacagcttccaacagggtggagggatctcgccagagtctgagcaccactgagctatagaatgtgtgggctgaactggtcctagcacccaacctatggtacaggtggggaaactgggaccagcgagggctaaggacttggcctcttgtccctgtcttttctgcctttcagtggtggagatgggcttcagggtgtagccaagcggtggctgggtggtgaggatgaggcctgacagctccctgtgcccccatagctccccctctctctgttcagtcctccctcgccacacgggggtggaagtgctcagcaggggctggcatcagggtttgcatggatccctagatgcacccccttccttgtctgtgaaacgaggggttcaggccagcccagggccccaatctttgattgcttacccatcaggaagctattgtctcccatacaagttgtgtttattaattcctggccaaacgccattccaagtcaggctggtgaggtggaaagcgcttaagtgtcgaagccagacaggccagggctcagcacctgtctcctctgcttcctacctgggcgaggacttacatctcccaacctcaggtaactcatctgaaaaaagggcgtgaaagagacccccaccctgggaagactaagtgagacaacgcgtggagaacattgcacacgcgggcttaggtcaagtgcaacaaacctgcgttcatcaccggctctcactctgctctgggcaggcacaagctgaggggtttatggtgctggctctttcagcctcaacaacccagcgaggaagcaggtgcctgtactgccttcacagaccagtgagacacccaagacacagagagatgaagtaatttgcacaaagtcacccagctctttgagccagagttaaggccaggcagcctgatctggagtgcacgtgggtgcacagatgcatgtctgtgtgcgtgcgtacatccatgcatgtctgtgcacgtgtacgtgcatgtgtgtgtggtccacgtgtgcgattcttccctctgagcctctagcggcccatgccagctggtgactccctcagccaaggcatccccagccaacccactggcatctgggtggggggatcgacagtttctgtggctgtcccaccagttccagagcggcctgggaagtcccagccctttcttctcagactttcattaagggtccagggtccccaggggcagactcttgtcccctccccgcagactcctcctgtgtgaatgaatgtggaagggaaggcagaggtggcgcctgcaaaccatccgcactgggccactgtgccctctagttatgatcatgggcgatagtgatcatcccatgtagatgctgagaaattcttagaatgagcatttgttggaaatctgcttgtgtgggtggcaaagacatgagaggtctagggaagagcagattttcagacaaggcactttagggagggggaggtacagccctttggcccagaatgcccattgatggagagggcgggtcaggggagagggtatcttaaccctcaagtgccagcgtagtgatgaggaaaggctggcctggtgggccccccatggactaagcatccttaggcacttcacctgactcctctgagactgtggtgcctccttcacccctgacctgcctgctttctacctagcttctcccggtgcccacttgagcccagctgaggcctcaggcccttgagtggcctgggggtggtagagggacttggcccgtgagatctggccatggctgctccatttcgcagaagccactctcacgggctgccaccgaagcacgggcttccccctttccgggaacctgcctcctgccagcttcctctcctgtgacatcacttctcttgtgattcgccccaccatttccactcactcccagccagtggggacaggcagaaccatgggttccctaggccagctggagccacccccgacccggcctggcctggctatggggtggcccttgtgttctccggagcgctagtggccagcacaggcggcagccacagacacttagtaggaacttcagtgtggctgacctgagctgggctggccgtgcaggagagtgcaagctgcttcctccatgagctcacagcctgacgtcagcaagtgcttcaaagaagtcatttcctatgcatgccttaaaccatgccacaagggagatacgatcacccctgttttacaaatgtgaaaactaaagcttgctgagggtgacccaaggtcacacagcttgttcctggggcaaagccaggctgccaattcagctctgcagccccaggtctagagctctggcaatgccaggtgctgctctcctcccctcttcagcacttgccttctgtgaccctccttcccctttaatctgtctgtaggtaagggcacgggggtgtgcattcatccacccacgcacccttctttccttcttccttcttgtgttctccccacccttccatccatccatccatccatccatgcatctatccctccaggcagtacatcctgacagggtccctgtctacctcctggatgaggcaagaaggaaatattccccatatccagagaggtgaggaagcaaggcaggccacacggtgcaaaaatgtgccttcagacactcagtactttgtagccaagatgaactggcaggcatcgcagcagtcaggcttctggtgcttcttggagagggctagaggggagcacttgttggacgggaggcactggagagccagagaatgtgcaccctcccccagagagttctgcagcagaaacagaaaactcagatgggccaaggggccaggccagggctagagtctatgatggggggtagggtagtccagtggtgttttcggggcttttctttctttctctctttctctttctttctttctttctttctttctttctttctttctttctttttctttctttctttctctttttctccttctccttctccttcttcctcttctttctctttcttctttcttcttccttattctccttttcccttcttctcccttcctcttctccttcttctccttctcttccttctcctcctcctctttcttcttcttctccttctcctcttcctcctcctccttcttcttctcctcctccttctcctcattctctttctcctttcttcctcttcatcttttcttcttcttctcctccgcctcctccttcctcttcctcttcctcttcctcttctccttctaaaggagcaggaatctggattattatgtgaaattagctcgcgactcaatgaagcaatttctacatggtgcataaacagattgtctttacgctgagtgactccgcttgggccactagatttcagccgctgccttgaattcctctctggcgctttctaagcagacgcttgttccagggattccaccacctctacccgtgctccaggcctccagagtgagaaccaaacactgcccagacagacaggttcccgggtacacggtgaggccctggggaaaggttgctgccagctacagactggttctaggactctccctggaggttgagagaacttcctgtagcaggcacaggtgtctttgccttacagcccctgcccaaggcttgggtgacactacaggtcctcaacgcagttgcttctagggtgaaacgttccactcccctccaaccccggcttgggttccttctctgtctccccacaatctccctgtgactgtgggaagggacaccccaaggcccatgggatgcgcttgactcctcattccccgcactagtccttcccaacccctggctcccctgtctacttcctgaggtccttctgtgaggaaaacaatccatgataactttatagacaaacagacaccaaaacctgcgtttcctgggttttacaagagcaagagggccaggcttgctcaggggcgccccctggcggtgcctcgtcccccaccggccctgctgggctgggggaaccatggtcgggggtggcggctcccaacctgttctgcctcaggacccagtcactctccgcaaaatgactgagtaccctaaagagtttttgcttatacaggttatagatctatacttgcagcattagaaattgaaacaaaattttaaaatgtttattaattcttttaatataattataagcccattacacatttgaatataaataacattctatgaaaattagttgcatcctccaaaagtaaaaacatttagtgacaagagtgctgtcattttacatttttgtacatttctttaacaactggcttcacagactacaggcgggaccttcgaatctgcctccgagttcaatcagtcccgatgtcacacatcagtctctggaaaactcgcctgtcaccttatgagagaatgagggcaaaaaaggcaaatgatatctgagtgttactataaacatgacttttggacccccaggggtcccctgactgtgctttgagaactgctggttggtgtaagggtaagatcgtggtcactgtggccagatagacttaggggggtgccagagtctaggccaggcgtgtggaggacatggggcatgtagggggctcagacctcagagctcctgttgcagtgggaattcggagccctcccctcaagcaagctaggtgagctcttctgggtcctgaggcaagattctggctccaccttggctcctgcactcttgagcctcatctgtaaaatgggatgagagcaattcctccctccctgggtggaggtgctgcttgaacctcagaatccccgtgcaatgaggccttgtgatgccatagccaatgaggctcagccccagccacacacctggagatgttaaaacagcctcaaagctcatcttcagctgttcggtggctaaggaattgattaacttattgaacggttaagtgcttaccacattctagaagttctggggaagtgcctggcccttgggaatcatggccggctccgcagggtgttggatttgctgtgggatgtccccactggccttcaggggcattcctgatgctctctggatttccatctgctttctctgccaggggcattttcagctctccctgcagattttcaacctgcaccctgagtgtgtttcccccatctgcaaagcactctgatttgctctgtggagggcatttctatgagctgatgaagctgtccccatctgttctgcaagggtgtcccacctgggatgaaaaggaacccccggctgctgtggagggagggtcccactgtcctgggggagtggctgcacccactctgtgaagtcatgccgctgcccacttgctctgtggggtgaggtgcaccggactctctgcaggaggaacccctgggcccatgccctggagatgggagggctcctacctgttctctggtaggagagaaagactcagcctctctggagattcccccacctgctctgtttgaacaacggtatcttcttggtggtggtatggcaggggtgcaggggcggtgttgtccagcagggatgtgagggtgctcccacagctgggggtggtcccaccccgtgtggccatgcacagagaaggtgctgcccatcagcactaagctactggtcatgggagaaggactggtccttccctcaagcccacagtgtcacagggaggcaggagggttggtgcctaaatggggagcactgctgccccctcgtcccacaccaagctcaaggcagatgaccgtgcacatctgtggacagtggggcagtcaagggcttttgcctcaactgacacattgaagccttttgtcagattcaagatcaacagaaataatttttcctttctttctttctctttctttcttttcttttcttttttctttccctccctctctccctttctttctttctctttctctttcttctttctttctttcttcctttctttctctttctttctttctttttccctccctcccttccttccttctttccctccctccttccttcctaccttctgtctctttctttctttttttgacgtactttcgttcttattgcccaggctggagtgcaatggcacgatctcggctcaccgcaacctctgcttcctgggttcaagcgattctcctgcttcagcctcccgagtagctgggattacaagcatgtgccaccatgcctggctaattttgtatttttagtagcaacggggtttctccatgttggtcagtctggtctcgaactcccgacttcaggtgatccacccacctcagcctcccaaagtgctgggattataggtgtgagccactgcgcccagccaatttttcttgttttataagggaggaaggtgaggctcaaagaaggaccctgacttgctagaacctcacagttcacaggtgactgtgactagaattgagttttttatctggcaggcaatggggagccattgaagatttttgagcagggcagtggcatagccaggctagtttctagaagatgactctgggggtgcactcatctaagggagaaatcagggcagaggaggcacagcgggcgtgcagctccccctgcccctctggctgcctgtccttgctctgtctgtgcacgggacccaggagaccagccagtgcagccctgagtcgtctctgactccccccaggctgtgtggcttgcgcatcctgcagccctacgccgagaggatccccgtggtggccacggccgggatcaccatcaacttcacctcccagatctccctcaccgggcccggtgtgcgggtgcactatggcttgtacaaccagtcggaccgtgagtatgggcagccgggggaaccccctgcagtgactcgctgcctcttggccatccctggaaccaccaagggggctgtgggcagctgcttatgaggctgaacaaaaggagagagagagtgtgtgtgtgtgtgtatgtgcttgcacaaatttatgcagctttgtgtgcccacgtgtgcaaggcagccacaagggtttgcaggaatacacactcatacatatccacgtgtgtgttgtgtattctgtgtgtgtgtctggatatgtatgtctgcttggactgtgtacacaggtgcccaggaccacgtctgtgggtgcctgtccatgcgcgtgtgagtgaacaggtgcatgcgtgtctttgtgcgccttcgcggctacgcatggcctaatggcgccctgcctgcctccacggtcccctgtggttttgcagcctgccctggagagttcctctgttctgtgaatggactctgtgtccctgcctgtgatggggtcaaggactgccccaacggcctggatgagagaaactgcggtgagtaacccgcccgcgcatccctcctctccctgcccatcccttctccttcctcacctttcctgctctgagctgagtggagaccccacttctacatgcagcttccattatgagcacccaggaagtggggttctctcactgtgccggggtggcaaaatgagacagaccagcaatgcagcctccccgagaccacctcgtgggacagtggcagggagaagtggggagccaggtctcctgacttccagctcagggccatcacccccagcccctgtcccagccagccttccaggaaggaacagaatgggtgagggagatgtccccctcctctgccctgtcaaaggtttaaatatgtgggaagagggaagcgagatgttcatggtggggggatgatcctgccacggtgctgggggaggtacctcatattcagaaactgaacatctggcttcaagttctggctcagccaagtgaccttggacaagtcacctcatctgtttccaccagtgaaatggggtatctcacagggttgctgtgaaactttgggtgtaaaatagcagagaaagaggccgggcgcagtggctcatgcctgtaatcctagcactttgggaggcggagtcgagcggatcacctgaggtcaggagttcaagatcagcctggccaacatggtgaaaccccgtctctactaaaaatacaataattagctgggcgtggtagcaggagcctgtaattaatctcagctactcgggagtctgaggcaggagaatcgcttggacctgggaggttgcagtgagatcatgccatcgcactccagccttcgtgacaagagcgagacataaaaataaagtagcagagaaagagatttgtgattggtaacgtgcaatacagcacaccttctacaggcatcgccaagccccggctggctcctctggcttcctcccacctgtcccctctctgtgtccccacacagtttgcagagccacattccagtgcaaagaggacagcacatgcatctcactgcccaaggtctgtgatgggcagcctgattgtctcaacggcagcgacgaagagcagtgccaggaaggtagggcaggcctagccgagtgtctggagggacaccaaaggcagtctaggcctgctacatgcttcagcaaaagtttctagcttctcctctcaacacccaccaacccctctgtatttacatctgtatgtctgtccattcatccatccatccatccatccatccatccatccatccatccatccatcttctggtctccaatcaccgtctgtccattgattcatacagctacccatttatctatgcatctactgacctgtgcaaccatcaatctccctatcatcaaactgtcaatctacccatttattggtttggctgactactggtctatatggccactgttccatccatccatccatccatccatccatccacccacccatctacccacccacccatccacccatccatcatccatccgtccatcatccatccatccatcatccgtctatccatccatccatccatccatcatccatccatccacccatcgtccatccgtccatcatccatccatccatccatcatccatccatcatccatctatccatccatcatccttccacccatccgtcatccacccatcgatcatccatctgtccatcatccatccatacatcatccatctatccatccatccattcatccatccatcatccatgcatcatccatccatcatccatccatccatccatcatccgtctatccatccatccatcatccatccatccatccatcatccatccgtccatcatccatccatccatcatccatctatccatccatccatccgtccatcatccatccatccatcatccatccatcatccatccgtccatcacccatccatccatcatccatccatccatcatccatccatccatcatccatccgtccatcatccatccatccatcgtccatcatccatccatccatccatcatccatccatccatcatccatccatccatccatcatccatccattcatccatcatccatccattcatccatcatccatctgtccatcgtctatccatccatcatccatcatccatccatccatccatccatccatccatcatccatccatccatcatccatcaatccatcaatccatcatccatccatccatcatccatcgatccatcatccatccatccatgcacccatccatcatccatccatccatccatcatccatccattcatccatcatccatccatccatcatccatccatccatcatccatccatccatgcaaccatccatcatccatccatccatcatccatccatccatcatccatccatccatccatcatccatccatccattcatccatcatccatccatccatcatccgttcatccatcatccatccattcacccatcatccatccatccatcatccatccatcatccgtccatccatcatctgtccatcatccatccatccatcatccatccaaccatccatcatccatccatccaccatccatccattcatccgtcagccatccatccatccatgcacccatccatcatccatccatccatccatccatcatccatccatcatccatccatcatccacccatccatcatccatccatccatctacccatccatccacccatccatccacccatccactgatctccctagccccctgtctgtccactggtccttatatccacacgtttatccaaccttctagctgtctgtcagtctccctaatggaccaccactccacccattggcttgtctgctcagtcttctgtctgggtctatttatccatccatccatctacccatccaactgaccaactgaccaacacttgcaggctacccagcgataggcaaggtgcagtaaggaagtgagaataaaacagcagagatgcaggccctgccttccaaggctcatctgttagtaggaggatatgatgggtgactctcctgccttgtaggaagattggagggcagggaggaggtcagacatgaaaagcttcctggaggaggtaggtgtttggcccttggtgagagctaaaacttaaataggcaggaggaaaggagagaggcaaagaccaagtggtggagtggaaagttctttacagtgaagagcagggaggaaaatgtggacaaccgggcagggccagagcctgggagattgccaggctaggtgcggaccctggtctaaaagtggaggcacagttctgccttcaagttccacactggagggggaggcatgatcttgtggtcaggatctccagtctgagaatggagacaccactttgtgctcaataggccagtctgagtggaggggctgtggggggcggggggacatggcctgcttttaggagaccctaaaggagactcaggaaaagactctctagtcacctcctggctcttctggctccatcgttcctgcaccccactttggaaggtttccttggggctcagagacccaccttctgtgccctgcccccatcccctctgtcccaggggtgccatgtgggacattcaccttccagtgtgaggaccggagctgcgtgaagaagcccaacccgcagtgtgatgggcggcccgactgcagggacggctcggatgaggagcactgtggtgagccctgcctggctgccggggccctggagcttgggagggagggggtgcccacagcaggaagctggagggaaatctcactgttgtcccctggtctctctctatctcatcctctgcccccttgcctgggtcctgatggtctctccccctccatcattctcctgttctctgtctctccatctctttcctttgcccttcctctctgtctgcttctccccttcccctcctcctctgtccaccccaccacctgcccccatccccagactgtggcctccagggcccctccagccgcattgttggtggagctgtgtcctccgagggtgagtggccatggcaggccagcctccaggttcggggtcgacacatctgtgggggggccctcatcgctgaccgctgggtgataacagctgcccactgcttccaggaggacaggtgagcgggagggtgtgggggcctaggcagtaagagacaagggcagggaaggcccggtgggaggtgcactgtgtctgagctctttgcagatagagggaagggtggtggaccccccagacaggctactgtgatgtgagttctagtcctggctccaccaggaccttctgggtccccggacacattgttccacctctctgccatctacttttggtatcttgctttaagttgggccagtaattcattcattcatctcattcactcattcagcaacacttgtgctcctactatgtgccagggctgtgctagatgctggggattcagtaaaggacagaactgcccaacctggtcataagctatgacactccccgaggtgtgacacgaggtagcaggtggggctggggagcccccaggggacatctcatcaggcctcatggccatctttcccatctgcttggtgggctgaaacctcccccaatccacccccagacagatctgggctccagatcccgcccccaggccctgcacagggatccccttttgtatcctctctgggacgcagggcgctctgaccacctagctctctttaaccccatctcaggctccccactgccctcaggtagagggtagagacccgaaggctgcccatctgccacccaggcagctgactgccgcagtccaattcctccacgctcaactcccacccgctccccactaggacccaccagcctcagggaattcagagcagcctgggtctgtaaagcacacaggaaaaaagaaatctgtgtcgggggcctggcactgtgctacattttttagatacacggtcttattggattctctcaagaacattcgagtagaaaatgccattcccatttgcagatgaggtggcagaggcttagagaggcacacccatgtctagggagggatgaagctggggcgtggaacccaggcaggccgagtgggtgaaggctgaacgctgtaccaccagctaggcgaccttcagggagggaagggagggctgggtgtggagggcactgtcccgggcggggatctggctatcttgagggtccctggatggggagaggcagcttcctcccacctcacctcaccccaccccaccccaccccaccccaccccagcatggcctccacggtgctgtggaccgtgttcctgggcaaggtgtggcagaactcgcgctggcctggagaggtgtccttcaaggtgagccgcctgctcctgcacccgtaccacgaagaggacagccatgactacgacgtggcgctgctgcagctcgaccacccggtggtgcgctcggccgccgtgcgccccgtctgcctgcccgcgcgctcccacttcttcgagcccggcctgcactgctggattacgggctggggcgccttgcgcgagggcggtgagcagcggggacttgcggcgggaggcggagggagaccgtgcggatctgcgccgtaacacctggcctggagaagggcggggctgggggtcccggggctccaccccataggccctctagtgctgggattcaaattgggctgaattttacggtagaaaaccaccatttaatgcggcctgtaggcccctgcccctcccctcctagctcttcccttccttctggaagggcgttatgtgtggggcaaaggggcaggtctgggacgccactgcccacgtgcaagctccacctgctgttccttgggctgcaagggtggaaggctcttaattactagcactttccacatccaggctggattttaggggaacttgacttcatataatccacccaacagccctacgggcggatgctgtggccctattttatggatggagaaaccaaggctcagagacatgttgctgtaagtcacacagccagagaggactggagcaaagattagaacccagggctggctgcctccagagcccctgctcttcctgctactgctctcagaaacagggtctctcccctttctacgttcactgaccagagtccctggcggccaccgcacagttttggggacacagacccagctggcaaacctacagacatgccctgcagcgttagtgttggtggcttcaaaaatgtgtacagtgacttacaatctggaagcaggcggggccgcagagatattttaaggatggggaaactgaggctcagaggaacagtgacttacccaaggggatggcagtggtcatggcaaagcaaaggctggttcattcactattccttcactcattcagtcactcaatgacactttctgagcaccaagtacgtaccaggcgtggggttaggggaagggtacataaggatgaagagagaacattctcgggggagacagacagtggtaagagctgacatggatggggagatgcaggaacagtggagacacagaggaggctcctgcccagctagggtcaggggaggcttccaggggagggttgtttaagctgaggcctggaagatgagttggcaacattcagacaaaggggaaagacattcaggtgaagacacaggtgccaagacaggaagatgtgagaacatccgcagcctgccagaggggctgaggtggggggcaggcgtgcctgggcgaggagcaaccagaatggcagacagggccttgggcgaggagcaaccagaatggcagacagggccttgccggccagcataaggatcttaggccaggagttctccctcctacctgcaccttagaaccatacggggagtttcaagaaaaactgcgtatcaaggctccccgggggactgtgatatgcagccctcgtggagaagcgctagggcagactgcagagttggggcactgcagagttctaaggaaaccatgaagggatcagatgtgggcttcggagacatctgcaggtgctgtaacagagcagcgaggagccagccagagcccagaggtgcctcagcagacagaggtgggggacaagaagctggaggaagacactcatccacacgggcttttttcttttttcttttttttgtttttttgagacagagtttcgctcttgttgcccaggctggagtgcaatggcgcgatctcggctcggatccccctcctcccgggttcaagcggttctcctgcctcagcctcctgagtaactgggattacaggcatgtgccaccacacccagctaattttgtatttttagtacagacagggtttctccatgttggtcaagctggtctcaaactcttgacctcaggtgttccgtccgcctcagcctcccaaagtgctgggattacaggcatgagccaccgtgcccggccctccacatgggctttggtcgggggctgtcaccatgaaccccacagagaaagagctagaataaagtgacagggaggcagaggggcaggtgcgaccctagcaggggtaagggtgggcagagcaggagagaagtaggctcctgagatgcaaagggaataatgttagggagaatagagaacaggggctccaggctcctgagatctcacttctgcccttgaccacggacaggccccatcagcaacgctctgcagaaagtggatgtgcagttgatcccacaggacctgtgcagcgaggtctatcgctaccaggtgacgccacgcatgctgtgtgccggctaccgcaagggcaagaaggatgcctgtcaggtgagtcccccgggcatgggagggagagaggagggagaaaggatgctgcccacatcaccagggtctggccctttgctcacatcagcctgctgaagcctcccatcctcccagcaaggtggtgatggccacccctactttacagaagaggagactggggcttagaaaggttgaggagcttgcccaaggttgcagagccacagatcagaagagatgctgtgatgggcaggtgttaggctcaaacccagttctgctccttgcccaccacaaggcactaggcccagggtcccacagtgaggtggatgcatggaagaagaaaggggtgtcagccacagaagggaggcggaggcagagtgggggcgtggggacacagccacagttccaggaggtcccaggctggctggaggccggggagggctggcttgggctctctccatttagcaggcgaggggaaagcagagctttaagactgaacgtgactctggcacccagtcaattcccaacagtcaggacttaatccctatggctcttcacctggaaaagggggtgcccttaccctgcttcagtcctttctcctttccccctttcagggtgactcaggtggtccgctggtgtgcaaggcactcagtggccgctggttcctggcggggctggtcagctggggcctgggctgtggccggcctaactacttcggcgtctacacccgcatcacaggtgtgatcagctggatccagcaagtggtgacctgaggaactgcccccctgcaaagcagggcccacctcctggactcagagagcccagggcaactgccaagcagggggacaagtattctggcggggggtgggggagagagcaggccctgtggtggcaggaggtggcatcttgtctcgtccctgatgtctgctccagtgatggcaggaggatggagaagtgccagcagctgggggtcaagacgtcccctgaggacccaggcccacacccagcccttctgcctcccaattctctctcctccgtccccttcctccactgctgcctaatgcaaggcagtggctcagcagcaagaatgctggttctacatcccgaggagtgtctgaggtgcgccccactctgtacagaggctgtttgggcagccttgcctccagagagcagattccagcttcggaagcccctggtctaacttgggatctgggaatggaaggtgctcccatcggaggggaccctcagagccctggagactgccaggtgggcctgctgccactgtaagccaaaaggtggggaagtcctgactccagggtccttgccccacccctgcctgccacctgggccctcacagcccagaccctcactgggaggtgagctcagctgccctttggaataaagctgcctgatccaagccccgctgctggagtttgaatgggacccaggcaccagcctcatgcccttgactggagcagcccctgcttcctgctcagcctgtttgacaagtgtccagaaggccaaggtgggctcagtggcagtgggcgtggccactgagggctggggcctgcagggcagctgcccaggtcccagaagaaatgccaggaaggcaatcatttggggaccctcaggtcagagggatgtgaggagcaatcgtctccttttggaaccttaggaggaaactgaggctcagagaggcggttaagacatcctcatagtggcactgggggttaggagtggaggtggcatagactcctgtctcccagctccctgtctgccaaggccccgtccagtgcgacactcccttcctttgcattctttgagccactgaataaagccttgggctccaaccatgtgccagcactatgctggggccacaggggtgaaggacctggctcctgaccccaggagcagtggggatgatccagtgggaaggggccggaggggagcgtggactgggcaagtcaaggcaagctgcctggaggctgtgagacttgagctggggttcagaggtggtccaggtgggaatatccgggaaggatattccaggcagggaagagcacgtgcaaaggcacagtcccggaagaatgaggcacgctaggacccagcaagccgagtgagtgttagaacagagctcgagaggatgactcaagaattcagaggggcgaactgaggcgggatagcagagcctggggttgagccaaggatttgatcttgaaagctctggggagccacggtgggctctatagcataggagtgacatgagaggattcacattttggaaccagccttggcaccagtgtgcagggagcggcaggcagggaggctggttaggaggccaccgcaggattccaggatggagaggatgggccgggactgagcagcgccatgggatggactggaggatgattttagacccctgggggcagttgtgatggaggcagggggctcgctggaggtgagggtggacggtcaagtgtggacaactctttctagacgcctaactgggagcggaagggagagagggagcttcagaggggccccagactgaagaggggtttttccaacatgggcgctgctgccaggtctgtgggtgaatgaggcagaaggggaaccagggacggggagcacccacctgggtcctgccaggacgagccggagcagctgggtgggcagggagcgtctccagagcaggtgggcagaacacatgcagaataccttgggtgatctggaatcaccctgggccctacctcagtcttcatcggaatcctggagggcgggggacgtgtcatctgttctcctaacaagcctcctggtgactcttttgcaaggatagttggaccctaaaaatgagtccagctttggagtggagtgtcctcaggggaagtggcgaggccctccaggcttgagctggcaagagggtgcccccgccccagcctgtggaaggcctgcgccttaggggctcactgcccggcaggatttcctcgagcagcggggaggactgaggagttgaaggaactggccagggtgggtggagggtctggggtctgggctgggtccagcagggtcagagaagggagagggcggggtgtttatatttcctaggattttgggcagaggggtggcagcaatagggagggatggcggtggcccaggtgtcagagtagaagtggagggggcgcgctgagaggtttaggatgtggcagaggcagcccagggctctccctagagttctgttttctggctcccggccaggtagggcaggtgctctggtatccggccccagggcaaaggatatagccagttccccaagccctccctgcaacacacacaggaaaatgacaacagggcagcgtccctgggcttttgggacaaagccgcgttcctttggaccagactaccacacctttagtttagccccgtccccaaaagtggcccagagaaagagggcaacagccaggctgggctgttcctttgggttttattacatggtggggtcggacacagctgagaagcaaggacccatcccgggaagtcaaacacaggagggcccctggctcagccgccatacccactctccccgggcagttcctgagtcctccaccgcccctgcccagccccttctgctgcctctccccgccccccaggccaggcgctgggccagcaatgcaaatggctgggggtgggatcaccaaagagaaggccaagccaactacccctactctgccaggccagctccccacaacctgcatccccaatacctgaatctccatttgcaaacacagtgttatgcccaggggtcgggctgggtccttcccatcccagggcagctgaaggtgggcggcccctatatactgcctgagggccttcagggactttgctcctctgtgcaccctcacaacaaccctgtgaggtaggtggggtgggaggagtgaccccctggactaaggctcaaggaggcaatgtgaccgggccaggaaggagcacatccaccatgcagcaggggagcccgggagaggggacgcaggtgccggagagacacagccagacattgccacacatctgccatgagcagtccactctgcccagaggtcctggggcccaccttgggccttaagaggtcccaggggggccccgccccgcccctggaggcaggagtaagtcacagccccacgggtgcagacagaggaggccggggagagggtgcttcttccttctcaggcccggggcccaccccatggtacaaaaataaaggatttcagatgggaaccccaagtccctggaggtgatctggggcctcacatccgggtgcctctggcttgtaacagctagaaaaaaaagaggggaagggcaggaggatgggaggggcggaggtggggccggtaaggagggggtgatgcagggcaagggggcggagaggagattgacgggtgggggagagggagagagagagaggcagttgagtcacaggcttccttctggaggagggggtggggctgaggcccaaagaaggtggattcagaactgagttggggggagcagcaagggctccccaactaacccatccaggagccccatgccccgtcttgggctcggtggcggccacctacagaggccagattctgccaagactctgaagggggtgggatgggggttgctcagggctgggagaggcactgatgccccaggcgaaagaagccacagggagcagctgtctgtcccaattttagaggcaattgtggcccagagagggacagtgacttgcccaaggtcacagagcaggcagaaaagagtgggatagggggcttgtgggcacatggccagggctttttctgccactctgcaatcctta

SEQ ID NO: 2 - DNA, 3209 bp, Homo sapien
cttgagccagacccagtccagctctggtgcctgccctctggtgcgagctgacctgagatgcacttccctcctctgtgagctgtctcggcacccacttgcagtcactgccgcctgatgttgttactcttccactccaaaaggatgcccgtggccgaggccccccaggtggctggcgggcagggggacggaggtgatggcgaggaagcggagccggaggggatgttcaaggcctgtgaggactccaagagaaaagcccggggctacctccgcctggtgcccctgtttgtgctgctggccctgctcgtgctggcttcggcgggggtgctactctggtatttcctagggtacaaggcggaggtgatggtcagccaggtgtactcaggcagtctgcgtgtactcaatcgccacttctcccaggatcttacccgccgggaatctagtgccttccgcagtgaaaccgccaaagcccagaagatgctcaaggagctcatcaccagcacccgcctgggaacttactacaactccagctccgtctattcctttggggagggacccctcacctgcttcttctggttcattctccaaatccccgagcaccgccggctgatgctgagccccgaggtggtgcaggcactgctggtggaggagctgctgtccacagtcaacagctcggctgccgtcccctacagggccgagtacgaagtggaccccgagggcctagtgatcctggaagccagtgtgaaagacatagctgcattgaattccacgctgggttgttaccgctacagctacgtgggccagggccaggtcctccggctgaaggggcctgaccacctggcctccagctgcctgtggcacctgcagggccccaaggacctcatgctcaaactccggctggagtggacgctggcagagtgccgggaccgactggccatgtatgacgtggccgggcccctggagaagaggctcatcacctcggtgtacggctgcagccgccaggagcccgtggtggaggttctggcgtcgggggccatcatggcggtcgtctggaagaagggcctgcacagctactacgaccccttcgtgctctccgtgcagccggtggtcttccaggcctgtgaagtgaacctgacgctggacaacaggctcgactcccagggcgtcctcagcaccccgtacttccccagctactactcgccccaaacccactgctcctggcacctcacggtgccctctctggactacggcttggccctctggtttgatgcctatgcactgaggaggcagaagtatgatttgccgtgcacccagggccagtggacgatccagaacaggaggctgtgtggcttgcgcatcctgcagccctacgccgagaggatccccgtggtggccacggccgggatcaccatcaacttcacctcccagatctccctcaccgggcccggtgtgcgggtgcactatggcttgtacaaccagtcggacccctgccctggagagttcctctgttctgtgaatggactctgtgtccctgcctgtgatggggtcaaggactgccccaacggcctggatgagagaaactgcgtttgcagagccacattccagtgcaaagaggacagcacatgcatctcactgcccaaggtctgtgatgggcagcctgattgtctcaacggcagcgacgaagagcagtgccaggaaggggtgccatgtgggacattcaccttccagtgtgaggaccggagctgcgtgaagaagcccaacccgcagtgtgatgggcggcccgactgcagggacggctcggatgaggagcactgtgactgtggcctccagggcccctccagccgcattgttggtggagctgtgtcctccgagggtgagtggccatggcaggccagcctccaggttcggggtcgacacatctgtgggggggccctcatcgctgaccgctgggtgataacagctgcccactgcttccaggaggacagcatggcctccacggtgctgtggaccgtgttcctgggcaaggtgtggcagaactcgcgctggcctggagaggtgtccttcaaggtgagccgcctgctcctgcacccgtaccacgaagaggacagccatgactacgacgtggcgctgctgcagctcgaccacccggtggtgcgctcggccgccgtgcgccccgtctgcctgcccgcgcgctcccacttcttcgagcccggcctgcactgctggattacgggctggggcgccttgcgcgagggcggccccatcagcaacgctctgcagaaagtggatgtgcagttgatcccacaggacctgtgcagcgaggtctatcgctaccaggtgacgccacgcatgctgtgtgccggctaccgcaagggcaagaaggatgcctgtcagggtgactcaggtggtccgctggtgtgcaaggcactcagtggccgctggttcctggcggggctggtcagctggggcctgggctgtggccggcctaactacttcggcgtctacacccgcatcacaggtgtgatcagctggatccagcaagtggtgacctgaggaactgcccccctgcaaagcagggcccacctcctggactcagagagcccagggcaactgccaagcagggggacaagtattctggcggggggtgggggagagagcaggccctgtggtggcaggaggtggcatcttgtctcgtccctgatgtctgctccagtgatggcaggaggatggagaagtgccagcagctgggggtcaagacgtcccctgaggacccaggcccacacccagcccttctgcctcccaattctctctcctccgtccccttcctccactgctgcctaatgcaaggcagtggctcagcagcaagaatgctggttctacatcccgaggagtgtctgaggtgcgccccactctgtacagaggctgtttgggcagccttgcctccagagagcagattccagcttcggaagcccctggtctaacttgggatctgggaatggaaggtgctcccatcggaggggaccctcagagccctggagactgccaggtgggcctgctgccactgtaagccaaaaggtggggaagtcctgactccagggtccttgccccacccctgcctgccacctgggccctcacagcccagaccctcactgggaggtgagctcagctgccctttggaataaagctgcctgatccaaaaaaaaaaaaaaaaa

SEQ ID NO: 3 - DNA, 20 bp, Artificial sequence
  Synthetic oligonucleotide
ctttattccaaagggcagct

SEQ ID NO: 4 - DNA, 20 bp, Artificial sequence
  Synthetic oligonucleotide
gcttagagtacagcccactt

SEQ ID NO: 5 - DNA, 20 bp, Artificial sequence
  Synthetic oligonucleotide
ccttccctgaaggttcctcc